European Patent Application EP 4 621 055 A1, published September 24, 2025. Title: 塩基配列差異の検出キット及び検出法. Applicant: 国立大学法人弘前大学. Application JP. The sequence listing filed with the application follows.

SEQUENCE LISTING (33 sequences)

SEQ ID NO: 1 - RNA, 21 nt, synthetic construct
  source 1..21: mol_type = other RNA
cagtttggccagcccaaaatc

SEQ ID NO: 2 - DNA, 22 bp, synthetic construct
  source 1..22: mol_type = other DNA
gcctttccattctttggatcag

SEQ ID NO: 3 - DNA, 22 bp, synthetic construct
  source 1..22: mol_type = other DNA
ctgcagggagagactgaaacct

SEQ ID NO: 4 - RNA, 18 nt, synthetic construct
  source 1..18: mol_type = other RNA
ggcatgagctgcgtgatg

SEQ ID NO: 5 - RNA, 19 nt, synthetic construct
  source 1..19: mol_type = other RNA
gtggcgtaggcaagagtgc

SEQ ID NO: 6 - DNA, 23 bp, synthetic construct
  source 1..23: mol_type = other DNA
ggtactggtggagtatttgatag

SEQ ID NO: 7 - DNA, 26 bp, synthetic construct
  source 1..26: mol_type = other DNA
cttccaatcaaaatgcacagagagtg

SEQ ID NO: 8 - DNA, 230 bp, synthetic construct
  source 1..230: mol_type = other DNA
gcatgaactacttggaggaccgtcgcttggtgcaccgcgacctggcagccaggaacgtactggtgaaaacaccgcagcatgtcaagatcacagattttgggctggccaaactgctgggtgcggaagagaaagaataccatgcagaaggaggcaaagtaaggaggtggctttaggtcagccagcattttcctgacaccagggaccaggctgccttcccactagctgtattg

SEQ ID NO: 9 - DNA, 20 bp, synthetic construct
  source 1..20: mol_type = other DNA
gcatgaactacttggaggac

SEQ ID NO: 10 - DNA, 20 bp, synthetic construct
  source 1..20: mol_type = other DNA
caatacagctagtgggaagg

SEQ ID NO: 11 - RNA, 17 nt, synthetic construct
  source 1..17: mol_type = other RNA
ccagcccaaaatctgtg

SEQ ID NO: 12 - DNA, 15 bp, synthetic construct
  source 1..15: mol_type = other DNA
acagattttgggcgg

SEQ ID NO: 13 - DNA, 15 bp, synthetic construct
  source 1..15: mol_type = other DNA
ccgcccaaaatctgt

SEQ ID NO: 14 - DNA, 16 bp, synthetic construct
  source 1..16: mol_type = other DNA
ccgcccaaaatctgtg

SEQ ID NO: 15 - DNA, 18 bp, synthetic construct
  source 1..18: mol_type = other DNA
tttggcccgcccaaaatc

SEQ ID NO: 16 - RNA, 21 nt, synthetic construct
  source 1..21: mol_type = other RNA
cagtttggccagcccaaaatc

SEQ ID NO: 17 - RNA, 21 nt, synthetic construct
  source 1..21: mol_type = other RNA
cagtttggccagcccaaaatc

SEQ ID NO: 18 - RNA, 21 nt, synthetic construct
  source 1..21: mol_type = other RNA
gattttgggctggccaaactg

SEQ ID NO: 19 - DNA, 20 bp, synthetic construct
  source 1..20: mol_type = other DNA
gattccaatgccatccactt

SEQ ID NO: 20 - DNA, 21 bp, synthetic construct
  source 1..21: mol_type = other DNA
gattttgggctggccaaactg

SEQ ID NO: 21 - DNA, 21 bp, synthetic construct
  source 1..21: mol_type = other DNA
gattttgggcgggccaaactg

SEQ ID NO: 22 - DNA, 18 bp, synthetic construct
  source 1..18: mol_type = other DNA
catcacgcagctcatgcc

SEQ ID NO: 23 - DNA, 18 bp, synthetic construct
  source 1..18: mol_type = other DNA
catcatgcagctcatgcc

SEQ ID NO: 24 - DNA, 17 bp, synthetic construct
  source 1..17: mol_type = other DNA
cacagattttgggctgg

SEQ ID NO: 25 - DNA, 17 bp, synthetic construct
  source 1..17: mol_type = other DNA
cacagattttgggcggg

SEQ ID NO: 26 - DNA, 56 bp, synthetic construct
  source 1..56: mol_type = other DNA
gcatgtcaagatcacagattttgggctggccaaactgctgggtgcggaagagaaag

SEQ ID NO: 27 - DNA, 56 bp, synthetic construct
  source 1..56: mol_type = other DNA
gcatgtcaagatcacagattttgggcgggccaaactgctgggtgcggaagagaaag

SEQ ID NO: 28 - RNA, 21 nt, synthetic construct
  source 1..21: mol_type = other RNA
gattttgggctggccaaactg

SEQ ID NO: 29 - RNA, 21 nt, synthetic construct
  source 1..21: mol_type = other RNA
gattttgggcgggccaaactg

SEQ ID NO: 30 - DNA, 19 bp, synthetic construct
  source 1..19: mol_type = other DNA
gtggcgtaggcaagagtgc

SEQ ID NO: 31 - DNA, 19 bp, synthetic construct
  source 1..19: mol_type = other DNA
gtgacgtaggcaagagtgc

SEQ ID NO: 32 - DNA, 23 bp, synthetic construct
  source 1..23: mol_type = other DNA
cttcacagccctgcgtaaacgtc

SEQ ID NO: 33 - DNA, 23 bp, synthetic construct
  source 1..23: mol_type = other DNA
gctccttatctcccctccccgta